European Patent Application EP 4 663 655 A2, published December 17, 2025. Title: Cardiac troponin I specific antibody, kit and uses thereof. Applicant: SHENZHEN MINDRAY BIO-MEDICAL ELECTRONICS CO., LTD. The sequence listing filed with the application follows.

SEQUENCE LISTING (84 sequences)

SEQ ID NO: 1 - protein, 6 aa, synthetic construct
SSYWMC

SEQ ID NO: 2 - protein, 5 aa, synthetic construct
GNPMC

SEQ ID NO: 3 - protein, 5 aa, synthetic construct
SSVMC

SEQ ID NO: 4 - protein, 5 aa, synthetic construct
YKYMC

SEQ ID NO: 5 - protein, 5 aa, synthetic construct
NYYMV

SEQ ID NO: 6 - protein, 5 aa, synthetic construct
NYDMA

SEQ ID NO: 7 - protein, 5 aa, synthetic construct
DYWMS

SEQ ID NO: 8 - protein, 5 aa, synthetic construct
NNYMS

SEQ ID NO: 9 - protein, 5 aa, synthetic construct
DTGVN

SEQ ID NO: 10 - protein, 5 aa, synthetic construct
DYSVT

SEQ ID NO: 11 - protein, 5 aa, synthetic construct
SKYIN

SEQ ID NO: 12 - protein, 18 aa, synthetic construct
CIYGGRSGSTYYANWLNG

SEQ ID NO: 13 - protein, 17 aa, synthetic construct
CISSFSNNNDYANWAKG

SEQ ID NO: 14 - protein, 17 aa, synthetic construct
CVHGGDGSTDYATWAKG

SEQ ID NO: 15 - protein, 18 aa, synthetic construct
CIFAGLFDNIYYTTWARG

SEQ ID NO: 16 - protein, 17 aa, synthetic construct
SISDDGGSTYYRDSVKG

SEQ ID NO: 17 - protein, 17 aa, synthetic construct
SISHGGNDTAYRDSVEG

SEQ ID NO: 18 - protein, 17 aa, synthetic construct
DIKYDGSSTNYAPSLLN

SEQ ID NO: 19 - protein, 17 aa, synthetic construct
IINLGTGETSYNVKFTG

SEQ ID NO: 20 - protein, 16 aa, synthetic construct
AIWSGGDTDYNSTLKS

SEQ ID NO: 21 - protein, 16 aa, synthetic construct
TRYPSGTTYDADSVKG

SEQ ID NO: 22 - protein, 17 aa, synthetic construct
GITTRSSNTAYSDSVKG

SEQ ID NO: 23 - protein, 13 aa, synthetic construct
ARRDDDGTHSLRL

SEQ ID NO: 24 - protein, 9 aa, synthetic construct
ARGLGDTNL

SEQ ID NO: 25 - protein, 6 aa, synthetic construct
TRDFDL

SEQ ID NO: 26 - protein, 10 aa, synthetic construct
ARDPAGATDL

SEQ ID NO: 27 - protein, 7 aa, synthetic construct
ATGGFDY

SEQ ID NO: 28 - protein, 9 aa, synthetic construct
TRGGYWFPY

SEQ ID NO: 29 - protein, 11 aa, synthetic construct
TRIGGTYYFDY

SEQ ID NO: 30 - protein, 14 aa, synthetic construct
ASLGIRGRNYVMYA

SEQ ID NO: 31 - protein, 10 aa, synthetic construct
ALLRGSRFDS

SEQ ID NO: 32 - protein, 6 aa, synthetic construct
IVGFFL

SEQ ID NO: 33 - protein, 7 aa, synthetic construct
ATSALTL

SEQ ID NO: 34 - protein, 11 aa, synthetic construct
QASERISIYLA

SEQ ID NO: 35 - protein, 13 aa, synthetic construct
QSSQSVHGSDWLS

SEQ ID NO: 36 - protein, 13 aa, synthetic construct
QSSQSVYNNNWLN

SEQ ID NO: 37 - protein, 13 aa, synthetic construct
QASQSVYDNRYLS

SEQ ID NO: 38 - protein, 16 aa, synthetic construct
RSSHSLLDSTGNTYLY

SEQ ID NO: 39 - protein, 16 aa, synthetic construct
RSSQSLIHRNGNIYLN

SEQ ID NO: 40 - protein, 16 aa, synthetic construct
RSSQSLEHPDGNTHLS

SEQ ID NO: 41 - protein, 16 aa, synthetic construct
RSSQSLVYSDGDTFLD

SEQ ID NO: 42 - protein, 16 aa, synthetic construct
RSSKNFVHSDGNTYLN

SEQ ID NO: 43 - protein, 16 aa, synthetic construct
RSSQSLLYTNGKKYLN

SEQ ID NO: 44 - protein, 16 aa, synthetic construct
RSSQSLLDTDGENYLN

SEQ ID NO: 45 - protein, 7 aa, synthetic construct
DTSKLAS

SEQ ID NO: 46 - protein, 7 aa, synthetic construct
TTSTLAS

SEQ ID NO: 47 - protein, 7 aa, synthetic construct
RASTLAS

SEQ ID NO: 48 - protein, 7 aa, synthetic construct
DASTLAS

SEQ ID NO: 49 - protein, 7 aa, synthetic construct
SVSNLGS

SEQ ID NO: 50 - protein, 7 aa, synthetic construct
RVSNRFS

SEQ ID NO: 51 - protein, 7 aa, synthetic construct
RVSNRFS

SEQ ID NO: 52 - protein, 7 aa, synthetic construct
EVSNRFS

SEQ ID NO: 53 - protein, 7 aa, synthetic construct
KVSNRLS

SEQ ID NO: 54 - protein, 7 aa, synthetic construct
YATNRDI

SEQ ID NO: 55 - protein, 7 aa, synthetic construct
DATKWAS

SEQ ID NO: 56 - protein, 11 aa, synthetic construct
CQSTYGIRDGN

SEQ ID NO: 57 - protein, 12 aa, synthetic construct
LGGYDTDIDTYG

SEQ ID NO: 58 - protein, 12 aa, synthetic construct
LAAYVDDGDTYG

SEQ ID NO: 59 - protein, 12 aa, synthetic construct
AGYKSYNDDDYG

SEQ ID NO: 60 - protein, 9 aa, synthetic construct
MEAPHGPFT

SEQ ID NO: 61 - protein, 9 aa, synthetic construct
LQGTHLPYT

SEQ ID NO: 62 - protein, 9 aa, synthetic construct
LQSTRFPYT

SEQ ID NO: 63 - protein, 9 aa, synthetic construct
FQATHFPFT

SEQ ID NO: 64 - protein, 9 aa, synthetic construct
GQVSKIPLT

SEQ ID NO: 65 - protein, 9 aa, synthetic construct
FQNLQSPYG

SEQ ID NO: 66 - protein, 9 aa, synthetic construct
WQSFKSPFD

SEQ ID NO: 67 - protein, 8 aa, synthetic construct
GIDLGSFA

SEQ ID NO: 68 - protein, 7 aa, synthetic construct
INSAGIL

SEQ ID NO: 69 - protein, 6 aa, synthetic construct
ARLYDL

SEQ ID NO: 70 - protein, 8 aa, synthetic construct
QSVYDNNA

SEQ ID NO: 71 - protein, 7 aa, synthetic construct
DASKLAS

SEQ ID NO: 72 - protein, 13 aa, synthetic construct
LGDYDCSSADCYA

SEQ ID NO: 73 - protein, 8 aa, synthetic construct
GIDLAGYA

SEQ ID NO: 74 - protein, 7 aa, synthetic construct
IASDGEK

SEQ ID NO: 75 - protein, 6 aa, synthetic construct
ARFYDL

SEQ ID NO: 76 - protein, 8 aa, synthetic construct
ESVYDNNA

SEQ ID NO: 77 - protein, 7 aa, synthetic construct
DASKVAS

SEQ ID NO: 78 - protein, 7 aa, synthetic construct
DASKVAS

SEQ ID NO: 79 - protein, 8 aa, synthetic construct
GIDLGSFA

SEQ ID NO: 80 - protein, 7 aa, synthetic construct
INSEDIL

SEQ ID NO: 81 - protein, 6 aa, synthetic construct
ARFWDL

SEQ ID NO: 82 - protein, 8 aa, synthetic construct
QSVYDGTA

SEQ ID NO: 83 - protein, 7 aa, synthetic construct
DASKLAS

SEQ ID NO: 84 - protein, 13 aa, synthetic construct
LGDYDCSSGDCYV